European Patent Application EP 4 501 952 A2, published February 5, 2025. Title: CONJUGATED HEPCIDIN MIMETICS. Applicant: Protagonist Therapeutics. Application US. The sequence listing filed with the application follows.

SEQUENCE LISTING (258 sequences)

SEQ ID NO: 1 - protein, 17 aa, synthetic construct
  REGION 1..17: note = Made in Lab - hepcidin analogue
  SITE 10: note = MISC_FEATURE - PEG11-Palm conjugated half-life extension moiety
DTHFPCIKFKPRSKGCK

SEQ ID NO: 2 - protein, 17 aa, synthetic construct
  REGION 1..17: note = Made in Lab - hepcidin analogue
  SITE 10: note = MISC_FEATURE - PEG11-Palm conjugated half-life extension moiety
  MOD_RES 15: note = Sarcosine
DTHFPCIKFKPRSKXCK

SEQ ID NO: 3 - protein, 16 aa, synthetic construct
  REGION 1..16: note = Made in Lab - hepcidin analogue
  SITE 10: note = MISC_FEATURE - PEG11-Palm conjugated half-life extension moiety
DTHFPCIKFKPRSKGC

SEQ ID NO: 4 - protein, 15 aa, synthetic construct
  REGION 1..15: note = Made in Lab - hepcidin analogue
  SITE 10: note = MISC_FEATURE - PEG11-Palm conjugated half-life extension moiety
DTHFPCIKFKPRSKC

SEQ ID NO: 5 - protein, 14 aa, synthetic construct
  REGION 1..14: note = Made in Lab - hepcidin analogue
  SITE 10: note = MISC_FEATURE - PEG11-Palm conjugated half-life extension moiety
DTHFPCIKFKPRSC

SEQ ID NO: 6 - protein, 13 aa, synthetic construct
  REGION 1..13: note = Made in Lab - hepcidin analogue
  SITE 10: note = MISC_FEATURE - PEG11-Palm conjugated half-life extension moiety
DTHFPCIKFKPRC

SEQ ID NO: 7 - protein, 12 aa, synthetic construct
  REGION 1..12: note = Made in Lab - hepcidin analogue
  SITE 10: note = MISC_FEATURE - PEG11-Palm conjugated half-life extension moiety
DTHFPCIKFKPC

SEQ ID NO: 8 - protein, 11 aa, synthetic construct
  REGION 1..11: note = Made in Lab - hepcidin analogue
  SITE 10: note = MISC_FEATURE - PEG11-Palm conjugated half-life extension moiety
DTHFPCIKFKC

SEQ ID NO: 9 - protein, 13 aa, synthetic construct
  REGION 1..13: note = Made in Lab - hepcidin analogue
  SITE 10: note = MISC_FEATURE - PEG11-Palm conjugated half-life extension moiety
DTHFPCIKFKPCK

SEQ ID NO: 10 - protein, 11 aa, synthetic construct
  REGION 1..11: note = Made in Lab - hepcidin analogue
  MOD_RES 8: note = D-form Lysine
  SITE 10: note = MISC_FEATURE - PEG11-Palm conjugated half-life extension moiety
DTHFPCIKFKC

SEQ ID NO: 11 - protein, 11 aa, synthetic construct
  REGION 1..11: note = Made in Lab - hepcidin analogue
  MOD_RES 8: note = Ornithine
  SITE 10: note = MISC_FEATURE - PEG11-Palm conjugated half-life extension moiety
DTHFPCIXFKC

SEQ ID NO: 12 - protein, 11 aa, synthetic construct
  REGION 1..11: note = Made in Lab - hepcidin analogue
  MOD_RES 8: note = Homoserine
  SITE 10: note = MISC_FEATURE - PEG11-Palm conjugated half-life extension moiety
DTHFPCIXFKC

SEQ ID NO: 13 - protein, 11 aa, synthetic construct
  REGION 1..11: note = Made in Lab - hepcidin analogue
  SITE 10: note = MISC_FEATURE - PEG11-Palm conjugated half-life extension moiety
DTHFPCIQFKC

SEQ ID NO: 14 - protein, 11 aa, synthetic construct
  REGION 1..11: note = Made in Lab - hepcidin analogue
  MOD_RES 8: note = ACETYLATION
  SITE 10: note = MISC_FEATURE - PEG11-Palm conjugated half-life extension moiety
DTHFPCIKFKC

SEQ ID NO: 15 - protein, 11 aa, synthetic construct
  REGION 1..11: note = Made in Lab - hepcidin analogue
  MOD_RES 8: note = Nle
  SITE 10: note = MISC_FEATURE - PEG11-Palm conjugated half-life extension moiety
DTHFPCIXFKC

SEQ ID NO: 16 - protein, 11 aa, synthetic construct
  REGION 1..11: note = Made in Lab - hepcidin analogue
  SITE 10: note = MISC_FEATURE - PEG11-Palm conjugated half-life extension moiety
DTHFPCIIFKC

SEQ ID NO: 17 - protein, 11 aa, synthetic construct
  REGION 1..11: note = Made in Lab - hepcidin analogue
  MOD_RES 9: note = N-Methyl-Phenylalanine
  SITE 10: note = MISC_FEATURE - PEG11-Palm conjugated half-life extension moiety
DTHFPCIKXKC

SEQ ID NO: 18 - protein, 11 aa, synthetic construct
  REGION 1..11: note = Made in Lab - hepcidin analogue
  MOD_RES 9: note = Alpha-Methyl-Phenylalanine
  SITE 10: note = MISC_FEATURE - PEG11-Palm conjugated half-life extension moiety
DTHFPCIKXKC

SEQ ID NO: 19 - protein, 11 aa, synthetic construct
  REGION 1..11: note = Made in Lab - hepcidin analogue
  MOD_RES 9: note = Beta homophenylalanine
  SITE 10: note = MISC_FEATURE - PEG11-Palm conjugated half-life extension moiety
DTHFPCIKXKC

SEQ ID NO: 20 - protein, 11 aa, synthetic construct
  REGION 1..11: note = Made in Lab - hepcidin analogue
  SITE 10: note = MISC_FEATURE - PEG11-Palm conjugated half-life extension moiety
DTHFPCIKWKC

SEQ ID NO: 21 - protein, 11 aa, synthetic construct
  REGION 1..11: note = Made in Lab - hepcidin analogue
  MOD_RES 8: note = D-form Lysine
  SITE 10: note = MISC_FEATURE - PEG8-Palm conjugated half-life extension moiety
DTHFPCIKFKC

SEQ ID NO: 22 - protein, 11 aa, synthetic construct
  REGION 1..11: note = Made in Lab - hepcidin analogue
  MOD_RES 8: note = D-form Lysine
  SITE 10: note = MISC_FEATURE - PEG4-Palm conjugated half-life extension moiety
DTHFPCIKFKC

SEQ ID NO: 23 - protein, 11 aa, synthetic construct
  REGION 1..11: note = Made in Lab - hepcidin analogue
  MOD_RES 8: note = D-form Lysine
  SITE 10: note = MISC_FEATURE - PEG2-Palm conjugated half-life extension moiety
DTHFPCIKFKC

SEQ ID NO: 24 - protein, 11 aa, synthetic construct
  REGION 1..11: note = Made in Lab - hepcidin analogue
  MOD_RES 8: note = D-form Lysine
  SITE 10: note = MISC_FEATURE - PEG1-Palm conjugated half-life extension moiety
DTHFPCIKFKC

SEQ ID NO: 25 - protein, 11 aa, synthetic construct
  REGION 1..11: note = Made in Lab - hepcidin analogue
  MOD_RES 8: note = D-form Lysine
  SITE 10: note = MISC_FEATURE - Aminohexanoic acid-palmityl conjugated half-life extension moiety
DTHFPCIKFKC

SEQ ID NO: 26 - protein, 11 aa, synthetic construct
  REGION 1..11: note = Made in Lab - hepcidin analogue
  MOD_RES 8: note = D-form Lysine
  SITE 10: note = MISC_FEATURE - PEG2-hexadecanoyl-gamma-Glu conjugated half-life extension moiety
DTHFPCIKFKC

SEQ ID NO: 27 - protein, 11 aa, synthetic construct
  REGION 1..11: note = Made in Lab - hepcidin analogue
  MOD_RES 8: note = D-form Lysine
  SITE 10: note = MISC_FEATURE - Hexadecanoyl-gamma-Glu conjugated half-life extension moiety
DTHFPCIKFKC

SEQ ID NO: 28 - protein, 11 aa, synthetic construct
  REGION 1..11: note = Made in Lab - hepcidin analogue
  MOD_RES 8: note = D-form Lysine
  SITE 10: note = MISC_FEATURE - IsoGlu-PEG2-Palm conjugated half-life extension moiety
DTHFPCIKFKC

SEQ ID NO: 29 - protein, 11 aa, synthetic construct
  REGION 1..11: note = Made in Lab - hepcidin analogue
  MOD_RES 8: note = D-form Lysine
  SITE 10: note = MISC_FEATURE - PEG2-Ahx-Palm conjugated half-life extension moiety
DTHFPCIKFKC

SEQ ID NO: 30 - protein, 11 aa, synthetic construct
  REGION 1..11: note = Made in Lab - hepcidin analogue
  MOD_RES 8: note = D-form Lysine
  SITE 10: note = MISC_FEATURE - Palm conjugated half-life extension moiety
DTHFPCIKFKC

SEQ ID NO: 31 - protein, 17 aa, synthetic construct
  REGION 1..17: note = Made in Lab - hepcidin analogue
  SITE 10: note = MISC_FEATURE - PEG11-Palm conjugated half-life extension moiety
  MOD_RES 15: note = Sarcosine
  MOD_RES 16: note = Penicillamine
DTHFPCIKFKPRSKXXK

SEQ ID NO: 32 - protein, 11 aa, synthetic construct
  REGION 1..11: note = Made in Lab - hepcidin analogue
  MOD_RES 8: note = D-form Lysine
  SITE 10: note = MISC_FEATURE - PEG11-Palm conjugated half-life extension moiety
  MOD_RES 11: note = Penicillamine
DTHFPCIKFKX

SEQ ID NO: 33 - protein, 11 aa, synthetic construct
  REGION 1..11: note = Made in Lab - hepcidin analogue
  MOD_RES 5: note = Nipecotic acid
  MOD_RES 8: note = D-form Lysine
  SITE 10: note = MISC_FEATURE - PEG11-Palm conjugated half-life extension moiety
DTHFXCIKFKC

SEQ ID NO: 34 - protein, 11 aa, synthetic construct
  REGION 1..11: note = Made in Lab - hepcidin analogue
  MOD_RES 5: note = D-form Nipecotic acid
  MOD_RES 8: note = D-form Lysine
  SITE 10: note = MISC_FEATURE - PEG11-Palm conjugated half-life extension moiety
DTHFXCIKFKC

SEQ ID NO: 35 - protein, 11 aa, synthetic construct
  REGION 1..11: note = Made in Lab - hepcidin analogue
  MOD_RES 5: note = D-form proline
  MOD_RES 8: note = D-form Lysine
  SITE 10: note = MISC_FEATURE - PEG11-Palm conjugated half-life extension moiety
DTHFPCIKFKC

SEQ ID NO: 36 - protein, 11 aa, synthetic construct
  REGION 1..11: note = Made in Lab - hepcidin analogue
  MOD_RES 5: note = D-form beta homoproline
  MOD_RES 8: note = D-form Lysine
  SITE 10: note = MISC_FEATURE - PEG11-Palm conjugated half-life extension moiety
DTHFXCIKFKC

SEQ ID NO: 37 - protein, 11 aa, synthetic construct
  REGION 1..11: note = Made in Lab - hepcidin analogue
  MOD_RES 5: note = beta homoproline
  MOD_RES 8: note = D-form Lysine
  SITE 10: note = MISC_FEATURE - PEG11-Palm conjugated half-life extension moiety
DTHFXCIKFKC

SEQ ID NO: 38 - protein, 11 aa, synthetic construct
  REGION 1..11: note = Made in Lab - hepcidin analogue
  MOD_RES 4: note = biphenylalanine
  MOD_RES 8: note = D-form Lysine
  SITE 10: note = MISC_FEATURE - PEG11-Palm conjugated half-life extension moiety
DTHXPCIKFKC

SEQ ID NO: 39 - protein, 11 aa, synthetic construct
  REGION 1..11: note = Made in Lab - hepcidin analogue
  MOD_RES 4: note = biphenylalanine
  MOD_RES 5: note = Nipecotic acid
  MOD_RES 8: note = D-form Lysine
  SITE 10: note = MISC_FEATURE - PEG11-Palm conjugated half-life extension moiety
DTHXXCIKFKC

SEQ ID NO: 40 - protein, 11 aa, synthetic construct
  REGION 1..11: note = Made in Lab - hepcidin analogue
  MOD_RES 5: note = Nipecotic acid
  MOD_RES 8: note = D-form Lysine
  SITE 10: note = MISC_FEATURE - PEG11-Palm conjugated half-life extension moiety
DTHFXCIKFKC

SEQ ID NO: 41 - protein, 17 aa, synthetic construct
  REGION 1..17: note = Made in Lab - hepcidin analogue
  MOD_RES 8: note = D-form lysine
  SITE 10: note = MISC_FEATURE - PEG11-Palm conjugated half-life extension moiety
  MOD_RES 15: note = Sarcosine
DTHFPCIKFKPRSKXCK

SEQ ID NO: 42 - protein, 17 aa, synthetic construct
  REGION 1..17: note = Made in Lab - hepcidin analogue
  MOD_RES 8: note = D-form lysine
  SITE 10: note = MISC_FEATURE - PEG11-Palm conjugated half-life extension moiety
  MOD_RES 15: note = Sarcosine
  MOD_RES 17: note = D-form lysine
DTHFPCIKFKPRSKXCK

SEQ ID NO: 43 - protein, 17 aa, synthetic construct
  REGION 1..17: note = Made in Lab - hepcidin analogue
  MOD_RES 8: note = D-form lysine
  SITE 10: note = MISC_FEATURE - PEG11-Palm conjugated half-life extension moiety
  MOD_RES 14: note = D-form lysine
  MOD_RES 15: note = Sarcosine
DTHFPCIKFKPRSKXCK

SEQ ID NO: 44 - protein, 17 aa, synthetic construct
  REGION 1..17: note = Made in Lab - hepcidin analogue
  MOD_RES 8: note = D-form lysine
  SITE 10: note = MISC_FEATURE - PEG11-Palm conjugated half-life extension moiety
  MOD_RES 13: note = D-form serine
  MOD_RES 15: note = Sarcosine
DTHFPCIKFKPRSKXCK

SEQ ID NO: 45 - protein, 17 aa, synthetic construct
  REGION 1..17: note = Made in Lab - hepcidin analogue
  MOD_RES 8: note = D-form lysine
  SITE 10: note = MISC_FEATURE - PEG11-Palm conjugated half-life extension moiety
  MOD_RES 12: note = D-form arginine
  MOD_RES 15: note = Sarcosine
DTHFPCIKFKPRSKXCK

SEQ ID NO: 46 - protein, 17 aa, synthetic construct
  REGION 1..17: note = Made in Lab - hepcidin analogue
  MOD_RES 8: note = D-form lysine
  SITE 10: note = MISC_FEATURE - PEG11-Palm conjugated half-life extension moiety
  MOD_RES 15: note = Sarcosine
  MOD_RES 17: note = D-form lysine
DTHFPCIKFKPRTKXCK

SEQ ID NO: 47 - protein, 17 aa, synthetic construct
  REGION 1..17: note = Made in Lab - hepcidin analogue
  MOD_RES 8: note = D-form lysine
  SITE 10: note = MISC_FEATURE - PEG11-Palm conjugated half-life extension moiety
  MOD_RES 15: note = Sarcosine
  MOD_RES 17: note = D-form lysine
DTHFPCIKFKPRTRXCK

SEQ ID NO: 48 - protein, 17 aa, synthetic construct
  REGION 1..17: note = Made in Lab - hepcidin analogue
  MOD_RES 8: note = D-form lysine
  SITE 10: note = MISC_FEATURE - PEG11-Palm conjugated half-life extension moiety
  MOD_RES 12: note = N-methylarginine
  MOD_RES 15: note = Sarcosine
  MOD_RES 17: note = D-form lysine
DTHFPCIKFKPXTKXCK

SEQ ID NO: 49 - protein, 17 aa, synthetic construct
  REGION 1..17: note = Made in Lab - hepcidin analogue
  MOD_RES 8: note = D-form lysine
  SITE 10: note = MISC_FEATURE - PEG11-Palm conjugated half-life extension moiety
  MOD_RES 12: note = D-form arginine
  MOD_RES 15: note = Sarcosine
  MOD_RES 17: note = D-form lysine
DTHFPCIKFKPRTKXCK

SEQ ID NO: 50 - protein, 17 aa, synthetic construct
  REGION 1..17: note = Made in Lab - hepcidin analogue
  MOD_RES 8: note = D-form lysine
  SITE 10: note = MISC_FEATURE - PEG11-Palm conjugated half-life extension moiety
  MOD_RES 15: note = Sarcosine
  MOD_RES 17: note = D-form lysine
DTHFPCIKFKPDTHXCK

SEQ ID NO: 51 - protein, 17 aa, synthetic construct
  REGION 1..17: note = Made in Lab - hepcidin analogue
  MOD_RES 8: note = D-form lysine
  SITE 10: note = MISC_FEATURE - PEG11-Palm conjugated half-life extension moiety
  MOD_RES 12: note = D-form arginine
  MOD_RES 14: note = N-methyllysine
  MOD_RES 15: note = Sarcosine
  MOD_RES 17: note = D-form lysine
DTHFPCIKFKPRTXXCK

SEQ ID NO: 52 - protein, 17 aa, synthetic construct
  REGION 1..17: note = Made in Lab - hepcidin analogue
  MOD_RES 8: note = D-form lysine
  SITE 10: note = MISC_FEATURE - PEG11-Palm conjugated half-life extension moiety
  MOD_RES 11: note = nipecotic acid
  MOD_RES 12: note = N-methylarginine
  MOD_RES 15: note = Sarcosine
  MOD_RES 17: note = D-form lysine
DTHFPCIKFKXXTHXCK

SEQ ID NO: 53 - protein, 17 aa, synthetic construct
  REGION 1..17: note = Made in Lab - hepcidin analogue
  SITE 10: note = MISC_FEATURE - PEG11-Palm conjugated half-life extension moiety
  SITE 15: note = misc_feature - Xaa can be any naturally occurring amino acid
  MOD_RES 16: note = Penicillamine
DTHFPCIKFKPRSKXXK

SEQ ID NO: 54 - protein, 11 aa, synthetic construct
  REGION 1..11: note = Made in Lab - hepcidin analogue
  MOD_RES 8: note = D-form lysine
  SITE 10: note = MISC_FEATURE - PEG11-Palm conjugated half-life extension moiety
  MOD_RES 11: note = Penicillamine
DTHFPCIKFKX

SEQ ID NO: 55 - protein, 18 aa, synthetic construct
  REGION 1..18: note = Made in Lab - hepcidin analogue
  MOD_RES 1: note = D-form lysine
  MOD_RES 2: note = D-form cysteine
  MOD_RES 3: note = Sarcosine
  MOD_RES 4: note = D-form lysine
  MOD_RES 5: note = D-form serine
  MOD_RES 6: note = D-form arginine
  MOD_RES 7: note = D-form proline
  MOD_RES 8: note = D-form lysine
  SITE 8: note = MISC_FEATURE - PEG11-Palm conjugated half-life extension moiety
  MOD_RES 9: note = D-form phenylalanine
  MOD_RES 10: note = D-form lysine
  MOD_RES 11: note = D-form isoleucine
  MOD_RES 12: note = D-form cysteine
  MOD_RES 13: note = D-form proline
  MOD_RES 14: note = D-form phenylalanine
  MOD_RES 15: note = D-form histidine
  MOD_RES 16: note = D-form threonine
  MOD_RES 17: note = D-form aspartic acid
  MOD_RES 18: note = D-form leucine
KCXKSRPKFKICPFHTDL

SEQ ID NO: 56 - protein, 11 aa, synthetic construct
  REGION 1..11: note = Made in Lab - hepcidin analogue
  MOD_RES 5: note = Nipecotic acid
  MOD_RES 8: note = D-form lysine
  SITE 10: note = MISC_FEATURE - PEG11-Palm conjugated half-life extension moiety
DTHFXCIKFKC

SEQ ID NO: 57 - protein, 11 aa, synthetic construct
  REGION 1..11: note = Made in Lab - hepcidin analogue
  MOD_RES 5: note = isoipecotic acid
  MOD_RES 8: note = D-form lysine
  SITE 10: note = MISC_FEATURE - PEG11-Palm conjugated half-life extension moiety
DTHFXCIKFKC

SEQ ID NO: 58 - protein, 11 aa, synthetic construct
  REGION 1..11: note = Made in Lab - hepcidin analogue
  MOD_RES 5: note = D-form proline
  MOD_RES 8: note = D-form lysine
  SITE 10: note = MISC_FEATURE - PEG11-Palm conjugated half-life extension moiety
DTHFPCIKFKC

SEQ ID NO: 59 - protein, 11 aa, synthetic construct
  REGION 1..11: note = Made in Lab - hepcidin analogue
  MOD_RES 5: note = D-form beta homoproline
  MOD_RES 8: note = D-form lysine
  SITE 10: note = MISC_FEATURE - PEG11-Palm conjugated half-life extension moiety
DTHFXCIKFKC

SEQ ID NO: 60 - protein, 11 aa, synthetic construct
  REGION 1..11: note = Made in Lab - hepcidin analogue
  MOD_RES 5: note = Beta homoproline
  MOD_RES 8: note = D-form lysine
  SITE 10: note = MISC_FEATURE - PEG11-Palm conjugated half-life extension moiety
DTHFXCIKFKC

SEQ ID NO: 61 - skipped

SEQ ID NO: 62 - protein, 11 aa, synthetic construct
  REGION 1..11: note = Made in Lab - hepcidin analogue
  MOD_RES 4: note = Biphenylalanine
  MOD_RES 8: note = D-form lysine
  SITE 10: note = MISC_FEATURE - PEG11-Palm conjugated half-life extension moiety
DTHXPCIKFKC

SEQ ID NO: 63 - protein, 11 aa, synthetic construct
  REGION 1..11: note = Made in Lab - hepcidin analogue
  MOD_RES 4: note = Biphenylalanine
  MOD_RES 5: note = Nipecotic acid
  MOD_RES 8: note = D-form lysine
  SITE 10: note = MISC_FEATURE - PEG11-Palm conjugated half-life extension moiety
DTHXXCIKFKC

SEQ ID NO: 64 - skipped

SEQ ID NO: 65 - protein, 11 aa, synthetic construct
  REGION 1..11: note = Made in Lab - hepcidin analogue
  MOD_RES 8: note = D-form lysine
  SITE 11: note = MISC_FEATURE - PEG11-Palm conjugated half-life extension moiety
DTHFPCIKFCK

SEQ ID NO: 66 - protein, 11 aa, synthetic construct
  REGION 1..11: note = Made in Lab - hepcidin analogue
  MOD_RES 5: note = Nipecotic acid
  MOD_RES 8: note = D-form lysine
  SITE 10: note = MISC_FEATURE - PEG11-Palm conjugated half-life extension moiety
DTHFXCIKFKC

SEQ ID NO: 67 - protein, 12 aa, synthetic construct
  REGION 1..12: note = Made in Lab - hepcidin analogue
  MOD_RES 6: note = Sulfhydryl (-SH) modification
  SITE 10: note = MISC_FEATURE - PEG11-Palm conjugated half-life extension moiety
  MOD_RES 12: note = Sulfhydryl (-SH) modification
DTHFPCIKFKPC

SEQ ID NO: 68 - protein, 11 aa, synthetic construct
  REGION 1..11: note = Made in Lab - hepcidin analogue
  MOD_RES 6: note = Sulfhydryl (-SH) modification
  MOD_RES 8: note = D-form lysine
  SITE 10: note = MISC_FEATURE - PEG11-Palm conjugated half-life extension moiety
  MOD_RES 11: note = Sulfhydryl (-SH) modification
DTHFPCIKFKC

SEQ ID NO: 69 - protein, 11 aa, synthetic construct
  REGION 1..11: note = Made in Lab - hepcidin analogue
  MOD_RES 6: note = Sulfhydryl (-SH) modification
  SITE 10: note = MISC_FEATURE - PEG11-Palm conjugated half-life extension moiety
  MOD_RES 11: note = Sulfhydryl (-SH) modification
DTHFPCIKFKC

SEQ ID NO: 70 - protein, 12 aa, synthetic construct
  REGION 1..12: note = Made in Lab - hepcidin analogue
  MOD_RES 8: note = D-form lysine
  SITE 10: note = MISC_FEATURE - PEG11-Palm conjugated half-life extension moiety
DTHFPCIKFKPC

SEQ ID NO: 71 - protein, 13 aa, synthetic construct
  REGION 1..13: note = Made in Lab - hepcidin analogue
  MOD_RES 8: note = D-form lysine
  SITE 10: note = MISC_FEATURE - PEG11-Palm conjugated half-life extension moiety
DTHFPCIKFKPRC

SEQ ID NO: 72 - protein, 14 aa, synthetic construct
  REGION 1..14: note = Made in Lab - hepcidin analogue
  MOD_RES 8: note = D-form lysine
  SITE 10: note = MISC_FEATURE - PEG11-Palm conjugated half-life extension moiety
DTHFPCIKFKPRSC

SEQ ID NO: 73 - protein, 15 aa, synthetic construct
  REGION 1..15: note = Made in Lab - hepcidin analogue
  MOD_RES 8: note = D-form lysine
  SITE 10: note = MISC_FEATURE - PEG11-Palm conjugated half-life extension moiety
DTHFPCIKFKPRSKC

SEQ ID NO: 74 - protein, 16 aa, synthetic construct
  REGION 1..16: note = Made in Lab - hepcidin analogue
  MOD_RES 8: note = D-form lysine
  SITE 10: note = MISC_FEATURE - PEG11-Palm conjugated half-life extension moiety
  MOD_RES 15: note = Sarcosine
DTHFPCIKFKPRSKXC

SEQ ID NO: 75 - protein, 16 aa, synthetic construct
  REGION 1..16: note = Made in Lab - hepcidin analogue
  MOD_RES 8: note = D-form lysine
  SITE 10: note = MISC_FEATURE - PEG11-Palm conjugated half-life extension moiety
DTHFPCIKFKPRSKCK

SEQ ID NO: 76 - protein, 16 aa, synthetic construct
  REGION 1..16: note = Made in Lab - hepcidin analogue
  MOD_RES 8: note = D-form lysine
  SITE 10: note = MISC_FEATURE - PEG11-Palm conjugated half-life extension moiety
DTHFPCIKFKPPRSCK

SEQ ID NO: 77 - protein, 14 aa, synthetic construct
  REGION 1..14: note = Made in Lab - hepcidin analogue
  MOD_RES 8: note = D-form lysine
  SITE 10: note = MISC_FEATURE - PEG11-Palm conjugated half-life extension moiety
DTHFPCIKFKPRCK

SEQ ID NO: 78 - protein, 12 aa, synthetic construct
  REGION 1..12: note = Made in Lab - hepcidin analogue
  MOD_RES 8: note = D-form lysine
  SITE 10: note = MISC_FEATURE - PEG11-Palm conjugated half-life extension moiety
DTHFPCIKFKCK

SEQ ID NO: 79 - protein, 12 aa, synthetic construct
  REGION 1..12: note = Made in Lab - hepcidin analogue
  MOD_RES 8: note = D-form lysine
  SITE 10: note = MISC_FEATURE - PEG11-Palm conjugated half-life extension moiety
DTHFPCIKFKRC

SEQ ID NO: 80 - protein, 12 aa, synthetic construct
  REGION 1..12: note = Made in Lab - hepcidin analogue
  MOD_RES 8: note = D-form lysine
  SITE 10: note = MISC_FEATURE - PEG11-Palm conjugated half-life extension moiety
DTHFPCIKFKKC

SEQ ID NO: 81 - protein, 12 aa, synthetic construct
  REGION 1..12: note = Made in Lab - hepcidin analogue
  MOD_RES 8: note = D-form lysine
  SITE 10: note = MISC_FEATURE - PEG11-Palm conjugated half-life extension moiety
  MOD_RES 11: note = D-form arginine
DTHFPCIKFKRC

SEQ ID NO: 82 - protein, 12 aa, synthetic construct
  REGION 1..12: note = Made in Lab - hepcidin analogue
  MOD_RES 8: note = D-form lysine
  SITE 10: note = MISC_FEATURE - PEG11-Palm conjugated half-life extension moiety
  MOD_RES 11: note = D-form lysine
DTHFPCIKFKKC

SEQ ID NO: 83 - protein, 13 aa, synthetic construct
  REGION 1..13: note = Made in Lab - hepcidin analogue
  MOD_RES 8: note = D-form lysine
  SITE 10: note = MISC_FEATURE - PEG11-Palm conjugated half-life extension moiety
  MOD_RES 13: note = D-form lysine
DTHFPCIKFKKCK

SEQ ID NO: 84 - protein, 13 aa, synthetic construct
  REGION 1..13: note = Made in Lab - hepcidin analogue
  MOD_RES 8: note = D-form lysine
  SITE 10: note = MISC_FEATURE - PEG11-Palm conjugated half-life extension moiety
  MOD_RES 13: note = D-form histidine
DTHFPCIKFKHCH

SEQ ID NO: 85 - protein, 13 aa, synthetic construct
  REGION 1..13: note = Made in Lab - hepcidin analogue
  MOD_RES 8: note = D-form lysine
  SITE 10: note = MISC_FEATURE - PEG11-Palm conjugated half-life extension moiety
  MOD_RES 13: note = D-form arginine
DTHFPCIKFKRCR

SEQ ID NO: 86 - protein, 12 aa, synthetic construct
  REGION 1..12: note = Made in Lab - hepcidin analogue
  MOD_RES 8: note = D-form lysine
  SITE 10: note = MISC_FEATURE - Ahx-Palm conjugated half-life extension moiety
DTHFPCIKFKKC

SEQ ID NO: 87 - protein, 12 aa, synthetic construct
  REGION 1..12: note = Made in Lab - hepcidin analogue
  MOD_RES 8: note = D-form lysine
  SITE 10: note = MISC_FEATURE - PEG2-Palm conjugated half-life extension moiety
DTHFPCIKFKKC

SEQ ID NO: 88 - protein, 12 aa, synthetic construct
  REGION 1..12: note = Made in Lab - hepcidin analogue
  MOD_RES 8: note = D-form lysine
  SITE 10: note = MISC_FEATURE - PEG2-PEG2-Palm conjugated half-life extension moiety
DTHFPCIKFKKC

SEQ ID NO: 89 - protein, 12 aa, synthetic construct
  REGION 1..12: note = Made in Lab - hepcidin analogue
  MOD_RES 8: note = D-form lysine
  SITE 10: note = MISC_FEATURE - PEG2-PEG2-C18 acid conjugated half-life extension moiety
DTHFPCIKFKKC

SEQ ID NO: 90 - protein, 12 aa, synthetic construct
  REGION 1..12: note = Made in Lab - hepcidin analogue
  MOD_RES 8: note = D-form lysine
  SITE 10: note = MISC_FEATURE - PEG2-PEG2-Ahx-Palm conjugated half-life extension moiety
DTHFPCIKFKKC

SEQ ID NO: 91 - protein, 12 aa, synthetic construct
  REGION 1..12: note = Made in Lab - hepcidin analogue
  MOD_RES 8: note = D-form lysine
  SITE 10: note = MISC_FEATURE - PEG4-Palm acid conjugated half-life extension moiety
DTHFPCIKFKKC

SEQ ID NO: 92 - protein, 12 aa, synthetic construct
  REGION 1..12: note = Made in Lab - hepcidin analogue
  MOD_RES 8: note = D-form lysine
  SITE 10: note = MISC_FEATURE - PEG4-Ahx-Palm conjugated half-life extension moiety
DTHFPCIKFKKC

SEQ ID NO: 93 - protein, 12 aa, synthetic construct
  REGION 1..12: note = Made in Lab - hepcidin analogue
  MOD_RES 8: note = D-form lysine
  SITE 10: note = MISC_FEATURE - PEG4-PEG4-Palm conjugated half-life extension moiety
DTHFPCIKFKKC

SEQ ID NO: 94 - protein, 12 aa, synthetic construct
  REGION 1..12: note = Made in Lab - hepcidin analogue
  MOD_RES 8: note = D-form lysine
  SITE 10: note = MISC_FEATURE - PEG4-isoGlu-Palm conjugated half-life extension moiety
DTHFPCIKFKKC

SEQ ID NO: 95 - protein, 12 aa, synthetic construct
  REGION 1..12: note = Made in Lab - hepcidin analogue
  MOD_RES 8: note = D-form lysine
  SITE 10: note = MISC_FEATURE - PEG8-Palm conjugated half-life extension moiety
DTHFPCIKFKKC

SEQ ID NO: 96 - protein, 12 aa, synthetic construct
  REGION 1..12: note = Made in Lab - hepcidin analogue
  MOD_RES 8: note = D-form lysine
  SITE 10: note = MISC_FEATURE - Behenic acid conjugated half-life extension moiety
DTHFPCIKFKKC

SEQ ID NO: 97 - protein, 12 aa, synthetic construct
  REGION 1..12: note = Made in Lab - hepcidin analogue
  MOD_RES 8: note = D-form lysine
  SITE 10: note = MISC_FEATURE - PEG11-Palm conjugated half-life extension moiety
  MOD_RES 12: note = D-form cysteine
DTHFPCIKFKKC

SEQ ID NO: 98 - protein, 12 aa, synthetic construct
  REGION 1..12: note = Made in Lab - hepcidin analogue
  MOD_RES 8: note = D-form lysine
  SITE 10: note = MISC_FEATURE - PEG11-Palm conjugated half-life extension moiety
  MOD_RES 12: note = Penicillamine
DTHFPCIKFKKC

SEQ ID NO: 99 - protein, 12 aa, synthetic construct
  REGION 1..12: note = Made in Lab - hepcidin analogue
  MOD_RES 8: note = D-form lysine
  SITE 10: note = MISC_FEATURE - PEG11-Palm conjugated half-life extension moiety
  MOD_RES 11: note = Diaminopropionic acid
DTHFPCIKFKXC

SEQ ID NO: 100 - protein, 12 aa, synthetic construct
  REGION 1..12: note = Made in Lab - hepcidin analogue
  MOD_RES 8: note = D-form lysine
  MOD_RES 9: note = beta,beta-diphenylalanine
  SITE 10: note = MISC_FEATURE - PEG11-Palm conjugated half-life extension moiety
DTHFPCIKXKKC

SEQ ID NO: 101 - protein, 12 aa, synthetic construct
  REGION 1..12: note = Made in Lab - hepcidin analogue
  MOD_RES 8: note = D-form lysine
  MOD_RES 9: note = Beta homophenylalanine
  SITE 10: note = MISC_FEATURE - PEG11-Palm conjugated half-life extension moiety
DTHFPCIKXKKC

SEQ ID NO: 102 - protein, 12 aa, synthetic construct
  REGION 1..12: note = Made in Lab - hepcidin analogue
  MOD_RES 8: note = D-form lysine
  MOD_RES 9: note = Napthylalanine
  SITE 10: note = MISC_FEATURE - PEG11-Palm conjugated half-life extension moiety
DTHFPCIKXKKC

SEQ ID NO: 103 - protein, 12 aa, synthetic construct
  REGION 1..12: note = Made in Lab - hepcidin analogue
  MOD_RES 8: note = D-form lysine
  MOD_RES 9: note = Beta homophenylalanine
  SITE 10: note = MISC_FEATURE - PEG11-Palm conjugated half-life extension moiety
DTHFPCIKXKKC

SEQ ID NO: 104 - protein, 12 aa, synthetic construct
  REGION 1..12: note = Made in Lab - hepcidin analogue
  MOD_RES 4: note = beta,beta-diphenylalanine
  MOD_RES 8: note = D-form lysine
  SITE 10: note = MISC_FEATURE - PEG11-Palm conjugated half-life extension moiety
DTHXPCIKFKKC

SEQ ID NO: 105 - protein, 12 aa, synthetic construct
  REGION 1..12: note = Made in Lab - hepcidin analogue
  MOD_RES 4: note = beta,beta-diphenylalanine
  MOD_RES 8: note = D-form lysine
  MOD_RES 9: note = Beta homophenylalanine
  SITE 10: note = MISC_FEATURE - PEG11-Palm conjugated half-life extension moiety
  MOD_RES 11: note = D-form lysine
DTHXPCIKXKKC

SEQ ID NO: 106 - protein, 11 aa, synthetic construct
  REGION 1..11: note = Made in Lab - hepcidin analogue
  SITE 9: note = MISC_FEATURE - PEG11-Palm conjugated half-life extension moiety
DTHFPCIFKKC

SEQ ID NO: 107 - protein, 12 aa, synthetic construct
  REGION 1..12: note = Made in Lab - hepcidin analogue
  MOD_RES 8: note = D-form lysine
  MOD_RES 10: note = D-form lysine
  SITE 10: note = MISC_FEATURE - PEG11-Palm conjugated half-life extension moiety
  MOD_RES 11: note = D-form lysine
DTHFPCIKFKKC

SEQ ID NO: 108 - skipped

SEQ ID NO: 109 - protein, 12 aa, synthetic construct
  REGION 1..12: note = Made in Lab - hepcidin analogue
  MOD_RES 4: note = beta,beta-diphenylalanine
  MOD_RES 5: note = Nipecotic acid
  MOD_RES 8: note = D-form lysine
  SITE 10: note = MISC_FEATURE - PEG11-Palm conjugated half-life extension moiety
DTHXXCIKFKKC

SEQ ID NO: 110 - protein, 12 aa, synthetic construct
  REGION 1..12: note = Made in Lab - hepcidin analogue
  MOD_RES 4: note = beta,beta-diphenylalanine
  MOD_RES 5: note = Nipecotic acid
  MOD_RES 8: note = D-form lysine
  MOD_RES 9: note = Phenylalanine (4-tBu)
  SITE 10: note = MISC_FEATURE - PEG11-Palm conjugated half-life extension moiety
DTHXXCIKXKKC

SEQ ID NO: 111 - protein, 12 aa, synthetic construct
  REGION 1..12: note = Made in Lab - hepcidin analogue
  MOD_RES 4: note = beta,beta-diphenylalanine
  MOD_RES 5: note = Nipecotic acid
  MOD_RES 8: note = D-form lysine
  MOD_RES 9: note = Phenylalanine (4-(2-aminoethoxy))
  SITE 10: note = MISC_FEATURE - PEG11-Palm conjugated half-life extension moiety
DTHXXCIKXKKC

SEQ ID NO: 112 - protein, 12 aa, synthetic construct
  REGION 1..12: note = Made in Lab - hepcidin analogue
  MOD_RES 4: note = beta,beta-diphenylalanine
  MOD_RES 5: note = Nipecotic acid
  MOD_RES 8: note = D-form lysine
  MOD_RES 9: note = 2-Napthylalanine
  SITE 10: note = MISC_FEATURE - PEG11-Palm conjugated half-life extension moiety
DTHXXCIKXKKC

SEQ ID NO: 113 - protein, 12 aa, synthetic construct
  REGION 1..12: note = Made in Lab - hepcidin analogue
  MOD_RES 4: note = beta,beta-diphenylalanine
  MOD_RES 5: note = Nipecotic acid
  MOD_RES 8: note = D-form lysine
  MOD_RES 9: note = Phenylalanine (4-COOOH)
  SITE 10: note = MISC_FEATURE - PEG11-Palm conjugated half-life extension moiety
DTHXXCIKXKKC

SEQ ID NO: 114 - protein, 12 aa, synthetic construct
  REGION 1..12: note = Made in Lab - hepcidin analogue
  MOD_RES 8: note = D-form lysine
  SITE 10: note = MISC_FEATURE - PEG11-Palm conjugated half-life extension moiety
  MOD_RES 12: note = Alpha-methylcysteine
DTHFPCIKFKKX

SEQ ID NO: 115 - protein, 12 aa, synthetic construct
  REGION 1..12: note = Made in Lab - hepcidin analogue
  MOD_RES 6: note = Alpha-methylcysteine
  MOD_RES 8: note = D-form lysine
  SITE 10: note = MISC_FEATURE - PEG11-Palm conjugated half-life extension moiety
  MOD_RES 12: note = Alpha-methylcysteine
DTHFPXIKFKKX

SEQ ID NO: 116 - protein, 12 aa, synthetic construct
  REGION 1..12: note = Made in Lab - hepcidin analogue
  MOD_RES 6: note = Alpha-methylcysteine
  MOD_RES 8: note = D-form lysine
  SITE 10: note = MISC_FEATURE - PEG11-Palm conjugated half-life extension moiety
DTHFPXIKFKKC

SEQ ID NO: 117 - protein, 12 aa, synthetic construct
  REGION 1..12: note = Made in Lab - hepcidin analogue
  MOD_RES 4: note = beta,beta-diphenylalanine
  MOD_RES 5: note = Nipecotic acid
  MOD_RES 8: note = D-form lysine
  SITE 10: note = MISC_FEATURE - PEG11-Palm conjugated half-life extension moiety
  MOD_RES 11: note = D-form lysine
DTHXXCIKFKKC

SEQ ID NO: 118 - protein, 12 aa, synthetic construct
  REGION 1..12: note = Made in Lab - hepcidin analogue
  MOD_RES 5: note = Nipecotic acid
  MOD_RES 8: note = D-form lysine
  SITE 10: note = MISC_FEATURE - PEG11-Palm conjugated half-life extension moiety
  MOD_RES 11: note = D-form lysine
DTHFXCIKFKKC

SEQ ID NO: 119 - protein, 12 aa, synthetic construct
  REGION 1..12: note = Made in Lab - hepcidin analogue
  MOD_RES 4: note = beta,beta-diphenylalanine
  MOD_RES 5: note = Beta-homoproline
  MOD_RES 8: note = D-form lysine
  SITE 10: note = MISC_FEATURE - PEG11-Palm conjugated half-life extension moiety
  MOD_RES 11: note = D-form lysine
DTHXXCIKFKKC

SEQ ID NO: 120 - protein, 12 aa, synthetic construct
  REGION 1..12: note = Made in Lab - hepcidin analogue
  MOD_RES 4: note = Phenylalanine (4-COOH)
  MOD_RES 8: note = D-form lysine
  SITE 10: note = MISC_FEATURE - PEG11-Palm conjugated half-life extension moiety
  MOD_RES 11: note = D-form lysine
DTHXPCIKFKKC

SEQ ID NO: 121 - protein, 12 aa, synthetic construct
  REGION 1..12: note = Made in Lab - hepcidin analogue
  MOD_RES 4: note = Beta-homophenylalanine
  MOD_RES 8: note = D-form lysine
  SITE 10: note = MISC_FEATURE - PEG11-Palm conjugated half-life extension moiety
  MOD_RES 11: note = D-form lysine
DTHXPCIKFKKC

SEQ ID NO: 122 - protein, 12 aa, synthetic construct
  REGION 1..12: note = Made in Lab - hepcidin analogue
  MOD_RES 4: note = beta,beta-diphenylalanine
  MOD_RES 8: note = D-form lysine
  MOD_RES 9: note = Beta-homophenylalanine
  SITE 10: note = MISC_FEATURE - PEG11-Palm conjugated half-life extension moiety
  MOD_RES 11: note = D-form lysine
DTHXPCIKXKKC

SEQ ID NO: 123-124 - skipped (2 entries)

SEQ ID NO: 125 - protein, 12 aa, synthetic construct
  REGION 1..12: note = Made in Lab - hepcidin analogue
  MOD_RES 4: note = beta,beta-diphenylalanine
  MOD_RES 5: note = Nipecotic acid
  MOD_RES 8: note = D-form lysine
  MOD_RES 9: note = Alpha-methylphenylalanine
  SITE 10: note = MISC_FEATURE - PEG11-Palm conjugated half-life extension moiety
DTHXXCIKXKKC

SEQ ID NO: 126 - protein, 12 aa, synthetic construct
  REGION 1..12: note = Made in Lab - hepcidin analogue
  MOD_RES 4: note = beta,beta-diphenylalanine
  MOD_RES 5: note = Nipecotic acid
  MOD_RES 8: note = D-form lysine
  MOD_RES 9: note = Phenylalanine (4-CN)
  SITE 10: note = MISC_FEATURE - PEG11-Palm conjugated half-life extension moiety
DTHXXCIKXKKC

SEQ ID NO: 127 - protein, 12 aa, synthetic construct
  REGION 1..12: note = Made in Lab - hepcidin analogue
  MOD_RES 4: note = beta,beta-diphenylalanine
  MOD_RES 5: note = Nipecotic acid
  MOD_RES 8: note = D-form lysine
  MOD_RES 9: note = Phenylalanine (3,4-diF)
  SITE 10: note = MISC_FEATURE - PEG11-Palm conjugated half-life extension moiety
DTHXXCIKXKKC

SEQ ID NO: 128 - protein, 12 aa, synthetic construct
  REGION 1..12: note = Made in Lab - hepcidin analogue
  MOD_RES 4: note = Alpha-methylphenylalanine
  MOD_RES 8: note = D-form lysine
  SITE 10: note = MISC_FEATURE - PEG11-Palm conjugated half-life extension moiety
  MOD_RES 11: note = D-form lysine
DTHXPCIKFKKC

SEQ ID NO: 129 - protein, 12 aa, synthetic construct
  REGION 1..12: note = Made in Lab - hepcidin analogue
  MOD_RES 4: note = Phenylalanine (4-(2-aminoethoxy))
  MOD_RES 8: note = D-form lysine
  SITE 10: note = MISC_FEATURE - PEG11-Palm conjugated half-life extension moiety
  MOD_RES 11: note = D-form lysine
DTHXPCIKFKKC

SEQ ID NO: 130 - protein, 12 aa, synthetic construct
  REGION 1..12: note = Made in Lab - hepcidin analogue
  MOD_RES 4: note = beta,beta-diphenylalanine
  MOD_RES 8: note = D-form lysine
  SITE 10: note = MISC_FEATURE - PEG11-Palm conjugated half-life extension moiety
  MOD_RES 11: note = D-form lysine
DIHXPCIKFKKC

SEQ ID NO: 131 - protein, 12 aa, synthetic construct
  REGION 1..12: note = Made in Lab - hepcidin analogue
  MOD_RES 4: note = beta,beta-diphenylalanine
  MOD_RES 8: note = D-form lysine
  MOD_RES 9: note = beta,beta-diphenylalanine
  SITE 10: note = MISC_FEATURE - PEG11-Palm conjugated half-life extension moiety
  MOD_RES 11: note = D-form lysine
DTHXPCIKXKKC

SEQ ID NO: 132 - protein, 12 aa, synthetic construct
  REGION 1..12: note = Made in Lab - hepcidin analogue
  MOD_RES 4: note = beta,beta-diphenylalanine
  MOD_RES 8: note = D-form lysine
  SITE 10: note = MISC_FEATURE - PEG11-Palm conjugated half-life extension moiety
  MOD_RES 11: note = D-form lysine
  MOD_RES 12: note = Penicillamine
DTHXPCIKFKKX

SEQ ID NO: 133 - protein, 12 aa, synthetic construct
  REGION 1..12: note = Made in Lab - hepcidin analogue
  MOD_RES 4: note = beta,beta-diphenylalanine
  MOD_RES 8: note = D-form lysine
  SITE 10: note = MISC_FEATURE - PEG11-Palm conjugated half-life extension moiety
  MOD_RES 12: note = N-methyl-cysteine
DTHXPCIKFKKX

SEQ ID NO: 134 - protein, 12 aa, synthetic construct
  REGION 1..12: note = Made in Lab - hepcidin analogue
  MOD_RES 4: note = beta,beta-diphenylalanine
  MOD_RES 8: note = D-form lysine
  SITE 10: note = MISC_FEATURE - PEG11-Palm conjugated half-life extension moiety
  MOD_RES 11: note = D-form lysine
  MOD_RES 12: note = N-methyl-cysteine
DTHXPCIKFKKX

SEQ ID NO: 135 - protein, 11 aa, synthetic construct
  REGION 1..11: note = Made in Lab - hepcidin analogue
  MOD_RES 4: note = beta,beta-diphenylalanine
  MOD_RES 8: note = D-form lysine
  SITE 10: note = MISC_FEATURE - PEG11-Palm conjugated half-life extension moiety
DTHXPCIKFKC

SEQ ID NO: 136 - protein, 12 aa, synthetic construct
  REGION 1..12: note = Made in Lab - hepcidin analogue
  MOD_RES 4: note = beta,beta-diphenylalanine
  MOD_RES 8: note = D-form lysine
  SITE 10: note = MISC_FEATURE - PEG11-Palm conjugated half-life extension moiety
  MOD_RES 11: note = Orn
DTHXPCIKFKXC

SEQ ID NO: 137 - protein, 12 aa, synthetic construct
  REGION 1..12: note = Made in Lab - hepcidin analogue
  MOD_RES 4: note = beta,beta-diphenylalanine
  MOD_RES 8: note = D-form lysine
  SITE 10: note = MISC_FEATURE - PEG11-Palm conjugated half-life extension moiety
  MOD_RES 11: note = Diaminobutyric acid
DTHXPCIKFKXC

SEQ ID NO: 138 - protein, 12 aa, synthetic construct
  REGION 1..12: note = Made in Lab - hepcidin analogue
  MOD_RES 4: note = beta,beta-diphenylalanine
  MOD_RES 8: note = D-form lysine
  SITE 10: note = MISC_FEATURE - PEG11-Palm conjugated half-life extension moiety
  MOD_RES 11: note = Beta-homolysine
DTHXPCIKFKXC

SEQ ID NO: 139 - protein, 12 aa, synthetic construct
  REGION 1..12: note = Made in Lab - hepcidin analogue
  MOD_RES 4: note = beta,beta-diphenylalanine
  MOD_RES 8: note = D-form lysine
  SITE 10: note = MISC_FEATURE - PEG11-Palm conjugated half-life extension moiety
  MOD_RES 11: note = D-form lysine
DTHXPCIKFKKC

SEQ ID NO: 140 - protein, 12 aa, synthetic construct
  REGION 1..12: note = Made in Lab - hepcidin analogue
  MOD_RES 4: note = beta,beta-diphenylalanine
  MOD_RES 8: note = D-form lysine
  SITE 10: note = MISC_FEATURE - PEG11-Palm conjugated half-life extension moiety
  MOD_RES 11: note = Diaminopropionic acid
  MOD_RES 12: note = Penicillamine
DTHXPCIKFKXX

SEQ ID NO: 141 - protein, 12 aa, synthetic construct
  REGION 1..12: note = Made in Lab - hepcidin analogue
  MOD_RES 4: note = beta,beta-diphenylalanine
  MOD_RES 6: note = Homocysteine
  MOD_RES 8: note = D-form lysine
  SITE 10: note = MISC_FEATURE - PEG11-Palm conjugated half-life extension moiety
  MOD_RES 11: note = Diaminopropionic acid
DTHXPXIKFKXC

SEQ ID NO: 142 - protein, 12 aa, synthetic construct
  REGION 1..12: note = Made in Lab - hepcidin analogue
  MOD_RES 4: note = beta,beta-diphenylalanine
  MOD_RES 6: note = Homocysteine
  MOD_RES 8: note = D-form lysine
  SITE 10: note = MISC_FEATURE - PEG11-Palm conjugated half-life extension moiety
  MOD_RES 11: note = Diaminopropionic acid
  MOD_RES 12: note = Homocystein
DTHXPXIKFKXX

SEQ ID NO: 143 - protein, 12 aa, synthetic construct
  REGION 1..12: note = Made in Lab - hepcidin analogue
  MOD_RES 4: note = beta,beta-diphenylalanine
  MOD_RES 8: note = D-form lysine
  SITE 10: note = MISC_FEATURE - PEG11-Palm conjugated half-life extension moiety
  MOD_RES 11: note = Diaminopropionic acid
  MOD_RES 12: note = Homocystein
DTHXPCIKFKXX

SEQ ID NO: 144 - protein, 12 aa, synthetic construct
  REGION 1..12: note = Made in Lab - hepcidin analogue
  MOD_RES 8: note = D-form lysine
  SITE 10: note = MISC_FEATURE - PEG11-Palm conjugated half-life extension moiety
DTHFPCIKFKCK

SEQ ID NO: 145 - protein, 12 aa, synthetic construct
  REGION 1..12: note = Made in Lab - hepcidin analogue
  MOD_RES 4: note = beta,beta-diphenylalanine
  MOD_RES 8: note = Beta-alanine
  MOD_RES 9: note = Beta-homophenylalanine
  SITE 10: note = MISC_FEATURE - PEG11-Palm conjugated half-life extension moiety
  MOD_RES 11: note = D-form lysine
DTHXPCIXXKKC

SEQ ID NO: 146 - protein, 12 aa, synthetic construct
  REGION 1..12: note = Made in Lab - hepcidin analogue
  MOD_RES 4: note = beta,beta-diphenylalanine
  MOD_RES 8: note = D-form alanine
  MOD_RES 9: note = Beta-homophenylalanine
  SITE 10: note = MISC_FEATURE - PEG11-Palm conjugated half-life extension moiety
  MOD_RES 11: note = D-form lysine
DTHXPCIAXKKC

SEQ ID NO: 147 - protein, 12 aa, synthetic construct
  REGION 1..12: note = Made in Lab - hepcidin analogue
  MOD_RES 4: note = beta,beta-diphenylalanine
  MOD_RES 9: note = Beta-homophenylalanine
  SITE 10: note = MISC_FEATURE - PEG11-Palm conjugated half-life extension moiety
  MOD_RES 11: note = D-form lysine
DTHXPCIIXKKC

SEQ ID NO: 148 - protein, 11 aa, synthetic construct
  REGION 1..11: note = Made in Lab - hepcidin analogue
  MOD_RES 4: note = beta,beta-diphenylalanine
  MOD_RES 8: note = Beta-homophenylalanine
  SITE 9: note = MISC_FEATURE - PEG11-Palm conjugated half-life extension moiety
  MOD_RES 10: note = D-form lysine
DTHXPCIXKKC

SEQ ID NO: 149 - protein, 12 aa, synthetic construct
  REGION 1..12: note = Made in Lab - hepcidin analogue
  MOD_RES 4: note = beta,beta-diphenylalanine
  MOD_RES 5: note = Nipecotic acid
  MOD_RES 8: note = D-form lysine
  MOD_RES 9: note = Phenylalanine (4-tButyl)
  SITE 10: note = MISC_FEATURE - PEG11-Palm conjugated half-life extension moiety
  MOD_RES 11: note = D-form lysine
DTHXXCIKXKKC

SEQ ID NO: 150 - protein, 12 aa, synthetic construct
  REGION 1..12: note = Made in Lab - hepcidin analogue
  MOD_RES 4: note = beta,beta-diphenylalanine
  MOD_RES 5: note = Nipecotic acid
  MOD_RES 8: note = D-form lysine
  MOD_RES 9: note = Phenylalanine (4-tButyl)
  SITE 10: note = MISC_FEATURE - PEG11-Palm conjugated half-life extension moiety
  MOD_RES 12: note = D-form lysine
DTHXXCIKXKCK

SEQ ID NO: 151 - protein, 12 aa, synthetic construct
  REGION 1..12: note = Made in Lab - hepcidin analogue
  MOD_RES 4: note = beta,beta-diphenylalanine
  MOD_RES 8: note = D-form lysine
  MOD_RES 9: note = Beta-homophenylalanine
  SITE 10: note = MISC_FEATURE - Ahx-Palm conjugated half-life extension moiety
  MOD_RES 11: note = Diaminopropionic acid
  MOD_RES 12: note = N-methyl-cysteine
DTHXPCIKXKXX

SEQ ID NO: 152 - protein, 12 aa, synthetic construct
  REGION 1..12: note = Made in Lab - hepcidin analogue
  MOD_RES 4: note = beta,beta-diphenylalanine
  MOD_RES 8: note = D-form lysine
  MOD_RES 9: note = Beta-homophenylalanine
  MOD_RES 10: note = ACETYLATION
  MOD_RES 11: note = D-form lysine
DTHXPCIKXKKC

SEQ ID NO: 153 - protein, 12 aa, synthetic construct
  REGION 1..12: note = Made in Lab - hepcidin analogue
  MOD_RES 4: note = beta,beta-diphenylalanine
  MOD_RES 8: note = D-form lysine
  SITE 8: note = MISC_FEATURE - PEG11-OMe conjugated half-life extension moiety
  MOD_RES 9: note = Beta-homophenylalanine
  SITE 10: note = MISC_FEATURE - PEG11-Palm conjugated half-life extension moiety
  MOD_RES 11: note = D-form lysine
  SITE 11: note = MISC_FEATURE - PEG11-OMe conjugated half-life extension moiety
DTHXPCIKXKKC

SEQ ID NO: 154 - protein, 12 aa, synthetic construct
  REGION 1..12: note = Made in Lab - hepcidin analogue
  MOD_RES 4: note = beta,beta-diphenylalanine
  MOD_RES 8: note = D-form lysine
  MOD_RES 9: note = Beta-homophenylalanine
  SITE 10: note = MISC_FEATURE - PEG11 conjugated half-life extension moiety
  MOD_RES 11: note = D-form lysine
DTHXPCIKXKKC

SEQ ID NO: 155 - protein, 12 aa, synthetic construct
  REGION 1..12: note = Made in Lab - hepcidin analogue
  MOD_RES 4: note = beta,beta-diphenylalanine
  MOD_RES 8: note = D-form lysine
  MOD_RES 9: note = Beta-homophenylalanine
  SITE 10: note = MISC_FEATURE - PEG11-octane conjugated half-life extension moiety
  MOD_RES 11: note = D-form lysine
DTHXPCIKXKKC

SEQ ID NO: 156 - protein, 12 aa, synthetic construct
  REGION 1..12: note = Made in Lab - hepcidin analogue
  MOD_RES 4: note = beta,beta-diphenylalanine
  MOD_RES 8: note = D-form lysine
  MOD_RES 9: note = Beta-homophenylalanine
  SITE 10: note = MISC_FEATURE - PEG11-Lauryl conjugated half-life extension moiety
  MOD_RES 11: note = D-form lysine
DTHXPCIKXKKC

SEQ ID NO: 157 - protein, 12 aa, synthetic construct
  REGION 1..12: note = Made in Lab - hepcidin analogue
  MOD_RES 4: note = beta,beta-diphenylalanine
  MOD_RES 8: note = D-form lysine
  MOD_RES 9: note = Beta-homophenylalanine
  SITE 10: note = MISC_FEATURE - PEG11-OMe conjugated half-life extension moiety
  MOD_RES 11: note = D-form lysine
DTHXPCIKXKKC

SEQ ID NO: 158 - protein, 12 aa, synthetic construct
  REGION 1..12: note = Made in Lab - hepcidin analogue
  MOD_RES 4: note = beta,beta-diphenylalanine
  MOD_RES 8: note = D-form lysine
  MOD_RES 9: note = Beta-homophenylalanine
  SITE 10: note = MISC_FEATURE - IsoGlu-Palm conjugated half-life extension moiety
  MOD_RES 11: note = D-form lysine
DTHXPCIKXKKC

SEQ ID NO: 159 - protein, 12 aa, synthetic construct
  REGION 1..12: note = Made in Lab - hepcidin analogue
  MOD_RES 4: note = beta,beta-diphenylalanine
  MOD_RES 8: note = D-form lysine
  MOD_RES 8: note = ACETYLATION
  MOD_RES 9: note = Beta-homophenylalanine
  SITE 10: note = MISC_FEATURE - PEG11-Palm conjugated half-life extension moiety
  MOD_RES 11: note = D-form lysine
DTHXPCIKXKKC

SEQ ID NO: 160 - protein, 11 aa, synthetic construct
  REGION 1..11: note = Made in Lab - hepcidin analogue
  MOD_RES 4: note = beta,beta-diphenylalanine
  MOD_RES 8: note = D-form lysine
  MOD_RES 9: note = Beta-homophenylalanine
  SITE 10: note = MISC_FEATURE - Dap-Palm conjugated half-life extension moiety
DTHXPCIKXKC

SEQ ID NO: 161 - protein, 11 aa, synthetic construct
  REGION 1..11: note = Made in Lab - hepcidin analogue
  MOD_RES 4: note = beta,beta-diphenylalanine
  MOD_RES 8: note = D-form lysine
  MOD_RES 9: note = Beta-homophenylalanine
  SITE 10: note = MISC_FEATURE - D-form Dap-Palm conjugated half-life extension moiety
DTHXPCIKXKC

SEQ ID NO: 162 - protein, 11 aa, synthetic construct
  REGION 1..11: note = Made in Lab - hepcidin analogue
  MOD_RES 4: note = beta,beta-diphenylalanine
  MOD_RES 8: note = D-form lysine
  MOD_RES 9: note = Beta-homophenylalanine
  MOD_RES 10: note = Diaminopropionic acid
  SITE 10: note = MISC_FEATURE - Dap-Palm conjugated half-life extension moiety
DTHXPCIKXXC

SEQ ID NO: 163 - protein, 11 aa, synthetic construct
  REGION 1..11: note = Made in Lab - hepcidin analogue
  MOD_RES 4: note = beta,beta-diphenylalanine
  MOD_RES 8: note = D-form lysine
  MOD_RES 9: note = Beta-homophenylalanine
  MOD_RES 10: note = Diaminopropionic acid
  SITE 10: note = MISC_FEATURE - D-form Dap-Palm conjugated half-life extension moiety
DTHXPCIKXXC

SEQ ID NO: 164 - protein, 11 aa, synthetic construct
  REGION 1..11: note = Made in Lab - hepcidin analogue
  MOD_RES 4: note = beta,beta-diphenylalanine
  MOD_RES 8: note = D-form lysine
  MOD_RES 9: note = Beta-homophenylalanine
  MOD_RES 10: note = Diaminopropionic acid
  SITE 10: note = MISC_FEATURE - D-form Dap-Palm conjugated half-life extension moiety
DTHXPCIKXXC

SEQ ID NO: 165 - protein, 12 aa, synthetic construct
  REGION 1..12: note = Made in Lab - hepcidin analogue
  MOD_RES 4: note = beta,beta-diphenylalanine
  MOD_RES 8: note = D-form lysine
  MOD_RES 9: note = Beta-homophenylalanine
  SITE 10: note = MISC_FEATURE - Ahx-Palm conjugated half-life extension moiety
  MOD_RES 11: note = D-form lysine
DTHXPCIKXKKC

SEQ ID NO: 166 - protein, 12 aa, synthetic construct
  REGION 1..12: note = Made in Lab - hepcidin analogue
  MOD_RES 4: note = beta,beta-diphenylalanine
  MOD_RES 8: note = D-form lysine
  SITE 8: note = MISC_FEATURE - PEG11-OMe conjugated half-life extension moiety
  MOD_RES 9: note = Beta-homophenylalanine
  SITE 10: note = MISC_FEATURE - Ahx-Palm conjugated half-life extension moiety
  MOD_RES 11: note = D-form lysine
  SITE 11: note = MISC_FEATURE - PEG11-OMe conjugated half-life extension moiety
DTHXPCIKXKKC

SEQ ID NO: 167 - protein, 12 aa, synthetic construct
  REGION 1..12: note = Made in Lab - hepcidin analogue
  MOD_RES 4: note = beta,beta-diphenylalanine
  MOD_RES 5: note = D-form proline
  MOD_RES 8: note = D-form lysine
  SITE 10: note = MISC_FEATURE - PEG11-Palm conjugated half-life extension moiety
  MOD_RES 11: note = D-form lysine
DTHXPCIKFKKC

SEQ ID NO: 168 - protein, 12 aa, synthetic construct
  REGION 1..12: note = Made in Lab - hepcidin analogue
  MOD_RES 4: note = Beta-homophenylalanine
  MOD_RES 5: note = D-form proline
  MOD_RES 8: note = D-form lysine
  SITE 10: note = MISC_FEATURE - PEG11-Palm conjugated half-life extension moiety
  MOD_RES 11: note = D-form lysine
DTHXPCIKFKKC

SEQ ID NO: 169 - protein, 12 aa, synthetic construct
  REGION 1..12: note = Made in Lab - hepcidin analogue
  MOD_RES 1: note = D-form aspartic acid
  MOD_RES 4: note = beta,beta-diphenylalanine
  MOD_RES 8: note = D-form lysine
  MOD_RES 9: note = Beta-homophenylalanine
  SITE 10: note = MISC_FEATURE - PEG11-Palm conjugated half-life extension moiety
  MOD_RES 11: note = D-form lysine
DTHXPCIKXKKC

SEQ ID NO: 170 - protein, 12 aa, synthetic construct
  REGION 1..12: note = Made in Lab - hepcidin analogue
  MOD_RES 4: note = beta,beta-diphenylalanine
  MOD_RES 8: note = D-form lysine
  MOD_RES 9: note = Beta-homophenylalanine
  SITE 10: note = MISC_FEATURE - PEG11-Palm conjugated half-life extension moiety
  MOD_RES 12: note = D-form lysine
DTHXPCIKXKCK

SEQ ID NO: 171 - protein, 12 aa, synthetic construct
  REGION 1..12: note = Made in Lab - hepcidin analogue
  MOD_RES 4: note = Beta-homophenylalanine
  MOD_RES 8: note = D-form lysine
  SITE 10: note = MISC_FEATURE - PEG11-Palm conjugated half-life extension moiety
  MOD_RES 12: note = D-form lysine
DTHXPCIKFKCK

SEQ ID NO: 172 - protein, 12 aa, synthetic construct
  REGION 1..12: note = Made in Lab - hepcidin analogue
  MOD_RES 4: note = Beta-homophenylalanine
  MOD_RES 5: note = Nipecotic acid
  MOD_RES 8: note = D-form lysine
  SITE 10: note = MISC_FEATURE - PEG11-Palm conjugated half-life extension moiety
  MOD_RES 12: note = D-form lysine
DTHXXCIKFKCK

SEQ ID NO: 173 - protein, 12 aa, synthetic construct
  REGION 1..12: note = Made in Lab - hepcidin analogue
  MOD_RES 4: note = beta,beta-diphenylalanine
  MOD_RES 5: note = Nipecotic acid
  MOD_RES 8: note = D-form lysine
  MOD_RES 9: note = Beta-homophenylalanine
  SITE 10: note = MISC_FEATURE - PEG11-Palm conjugated half-life extension moiety
  MOD_RES 12: note = D-form lysine
DTHXXCIKXKCK

SEQ ID NO: 174 - protein, 12 aa, synthetic construct
  REGION 1..12: note = Made in Lab - hepcidin analogue
  MOD_RES 4: note = beta,beta-diphenylalanine
  MOD_RES 8: note = D-form glutamine
  MOD_RES 9: note = Beta-homophenylalanine
  SITE 10: note = MISC_FEATURE - PEG11-Palm conjugated half-life extension moiety
  MOD_RES 11: note = D-form lysine
DTHXPCIQXKKC

SEQ ID NO: 175 - protein, 12 aa, synthetic construct
  REGION 1..12: note = Made in Lab - hepcidin analogue
  MOD_RES 4: note = beta,beta-diphenylalanine
  MOD_RES 8: note = D-form lysine
  MOD_RES 9: note = Beta-homophenylalanine
  SITE 10: note = MISC_FEATURE - PEG11-Palm conjugated half-life extension moiety
  MOD_RES 11: note = D-form lysine
  MOD_RES 11: note = ACETYLATION
DTHXPCIKXKKC

SEQ ID NO: 176 - protein, 12 aa, synthetic construct
  REGION 1..12: note = Made in Lab - hepcidin analogue
  MOD_RES 4: note = Beta-homophenylalanine
  MOD_RES 5: note = D-form proline
  MOD_RES 8: note = D-form lysine
  MOD_RES 9: note = Beta-homophenylalanine
  SITE 10: note = MISC_FEATURE - PEG11-Palm conjugated half-life extension moiety
  MOD_RES 12: note = D-form lysine
DTHXPCIKXKCK

SEQ ID NO: 177 - protein, 12 aa, synthetic construct
  REGION 1..12: note = Made in Lab - hepcidin analogue
  MOD_RES 4: note = beta,beta-diphenylalanine
  MOD_RES 8: note = D-form lysine
  MOD_RES 9: note = Beta-homophenylalanine
  SITE 10: note = MISC_FEATURE - Ahx-Palm conjugated half-life extension moiety
DTHXPCIKXKRC

SEQ ID NO: 178 - protein, 12 aa, synthetic construct
  REGION 1..12: note = Made in Lab - hepcidin analogue
  MOD_RES 4: note = beta,beta-diphenylalanine
  MOD_RES 8: note = D-form lysine
  MOD_RES 9: note = N-Methylphenylalanine
  SITE 10: note = MISC_FEATURE - Ahx-Palm conjugated half-life extension moiety
  MOD_RES 11: note = D-form lysine
DTHXPCIKXKKC

SEQ ID NO: 179 - protein, 12 aa, synthetic construct
  REGION 1..12: note = Made in Lab - hepcidin analogue
  MOD_RES 4: note = beta,beta-diphenylalanine
  MOD_RES 6: note = N-Methycysteine
  MOD_RES 8: note = D-form lysine
  MOD_RES 9: note = Beta-Homophenylalanine
  SITE 10: note = MISC_FEATURE - Ahx-Palm conjugated half-life extension moiety
  MOD_RES 11: note = D-form lysine
DTHXPXIKXKKC

SEQ ID NO: 180 - protein, 12 aa, synthetic construct
  REGION 1..12: note = Made in Lab - hepcidin analogue
  MOD_RES 4: note = N-Methylphenylalanine
  MOD_RES 8: note = D-form lysine
  MOD_RES 9: note = Beta-homophenylalanine
  SITE 10: note = MISC_FEATURE - Ahx-Palm conjugated half-life extension moiety
  MOD_RES 11: note = D-form lysine
DTHXPCIKXKKC

SEQ ID NO: 181 - protein, 12 aa, synthetic construct
  REGION 1..12: note = Made in Lab - hepcidin analogue
  MOD_RES 4: note = beta,beta-diphenylalanine
  MOD_RES 8: note = D-form lysine
  MOD_RES 9: note = Beta-homophenylalanine
  SITE 10: note = MISC_FEATURE - Ahx-Palm conjugated half-life extension moiety
  MOD_RES 11: note = D-form lysine
  MOD_RES 12: note = N-Methylcysteine
DTHXPCIKXKKX

SEQ ID NO: 182 - protein, 12 aa, synthetic construct
  REGION 1..12: note = Made in Lab - hepcidin analogue
  MOD_RES 4: note = beta,beta-diphenylalanine
  MOD_RES 5: note = Nipecotic aCID
  MOD_RES 8: note = D-form lysine
  MOD_RES 9: note = Phenylalanine (4-tBu)
  MOD_RES 10: note = D-form lysine
  SITE 12: note = MISC_FEATURE - PEG11-Palm conjugated half-life extension moiety
DTHXXCIKXKCK

SEQ ID NO: 183 - protein, 13 aa, synthetic construct
  REGION 1..13: note = Made in Lab - hepcidin analogue
  SITE 8: note = MISC_FEATURE - isoGlu-Palm conjugated half-life extension moiety
DTHFPCIKFEPKC

SEQ ID NO: 184 - protein, 12 aa, synthetic construct
  REGION 1..12: note = Made in Lab - hepcidin analogue
  SITE 8: note = MISC_FEATURE - isoGlu-Palm conjugated half-life extension moiety
  MOD_RES 11: note = D-form lysine
DTHFPCIKFEKC

SEQ ID NO: 185 - protein, 11 aa, synthetic construct
  REGION 1..11: note = Made in Lab - hepcidin analogue
  MOD_RES 8: note = D-form lysine
  SITE 8: note = MISC_FEATURE - isoGlu-Palm conjugated half-life extension moiety
DTHFPCIKFGC

SEQ ID NO: 186 - protein, 17 aa, synthetic construct
  REGION 1..17: note = Made in Lab - hepcidin analogue
  SITE 8: note = MISC_FEATURE - isoGlu-Palm conjugated half-life extension moiety
DTHFPCIKFEPRSKGCK

SEQ ID NO: 187 - protein, 12 aa, synthetic construct
  REGION 1..12: note = Made in Lab - hepcidin analogue
  MOD_RES 8: note = D-form lysine
  SITE 10: note = MISC_FEATURE - PEG11-Palm conjugated half-life extension moiety
  MOD_RES 11: note = Ornithine
DTHFPCIKFKXC

SEQ ID NO: 188 - protein, 12 aa, synthetic construct
  REGION 1..12: note = Made in Lab - hepcidin analogue
  MOD_RES 8: note = D-form lysine
  SITE 10: note = MISC_FEATURE - PEG11-Palm conjugated half-life extension moiety
  MOD_RES 11: note = diaminobutyric acid
DTHFPCIKFKXC

SEQ ID NO: 189 - protein, 12 aa, synthetic construct
  REGION 1..12: note = Made in Lab - hepcidin analogue
  MOD_RES 8: note = D-form lysine
  SITE 10: note = MISC_FEATURE - PEG11-Palm conjugated half-life extension moiety
  MOD_RES 11: note = homolysine
DTHFPCIKFKXC

SEQ ID NO: 190 - skipped

SEQ ID NO: 191 - protein, 12 aa, synthetic construct
  REGION 1..12: note = Made in Lab - hepcidin analogue
  MOD_RES 4: note = beta,beta-diphenylalanine
  MOD_RES 8: note = D-form lysine
  MOD_RES 9: note = Beta-homophenylalanine
  SITE 10: note = MISC_FEATURE - PEG11-Palm conjugated half-life extension moiety
DTHXPCIKXKKC

SEQ ID NO: 192 - protein, 12 aa, synthetic construct
  REGION 1..12: note = Made in Lab - hepcidin analogue
  MOD_RES 8: note = D-form lysine
  MOD_RES 10: note = D-form lysine
  SITE 10: note = MISC_FEATURE - PEG11-Palm conjugated half-life extension moiety
DTHFPCIKFKKC

SEQ ID NO: 193-200 - skipped (8 entries)

SEQ ID NO: 201 - protein, 16 aa, synthetic construct
  REGION 1..16: note = Made in Lab - hepcidin analogue
  SITE 8: note = MISC_FEATURE - IsoGlu-Palm conjugated half-life extension moiety
DTHFPCIKFEPRSKGC

SEQ ID NO: 202 - protein, 15 aa, synthetic construct
  REGION 1..15: note = Made in Lab - hepcidin analogue
  SITE 8: note = MISC_FEATURE - IsoGlu-Palm conjugated half-life extension moiety
DTHFPCIKFEPRSKC

SEQ ID NO: 203 - protein, 14 aa, synthetic construct
  REGION 1..14: note = Made in Lab - hepcidin analogue
  SITE 8: note = MISC_FEATURE - IsoGlu-Palm conjugated half-life extension moiety
DTHFPCIKFEPRSC

SEQ ID NO: 204 - protein, 13 aa, synthetic construct
  REGION 1..13: note = Made in Lab - hepcidin analogue
  SITE 8: note = MISC_FEATURE - IsoGlu-Palm conjugated half-life extension moiety
DTHFPCIKFEPRC

SEQ ID NO: 205 - protein, 12 aa, synthetic construct
  REGION 1..12: note = Made in Lab - hepcidin analogue
  SITE 8: note = MISC_FEATURE - IsoGlu-Palm conjugated half-life extension moiety
DTHFPCIKFEPC

SEQ ID NO: 206 - protein, 11 aa, synthetic construct
  REGION 1..11: note = Made in Lab - hepcidin analogue
  SITE 8: note = MISC_FEATURE - IsoGlu-Palm conjugated half-life extension moiety
DTHFPCIKFEC

SEQ ID NO: 207 - protein, 10 aa, synthetic construct
  REGION 1..10: note = Made in Lab - hepcidin analogue
  SITE 8: note = MISC_FEATURE - IsoGlu-Palm conjugated half-life extension moiety
DTHFPCIKFC

SEQ ID NO: 208 - protein, 13 aa, synthetic construct
  REGION 1..13: note = Made in Lab - hepcidin analogue
  SITE 8: note = MISC_FEATURE - IsoGlu-Palm conjugated half-life extension moiety
DTHFPCIKFEPCK

SEQ ID NO: 209 - protein, 13 aa, synthetic construct
  REGION 1..13: note = Made in Lab - hepcidin analogue
  SITE 8: note = MISC_FEATURE - IsoGlu-Palm conjugated half-life extension moiety
  MOD_RES 13: note = D-form lysine
DTHFPCIKFEPCK

SEQ ID NO: 210 - protein, 11 aa, synthetic construct
  REGION 1..11: note = Made in Lab - hepcidin analogue
  SITE 8: note = MISC_FEATURE - IsoGlu-Palm conjugated half-life extension moiety
DTHFPCIKFCK

SEQ ID NO: 211 - protein, 12 aa, synthetic construct
  REGION 1..12: note = Made in Lab - hepcidin analogue
  SITE 8: note = MISC_FEATURE - IsoGlu-Palm conjugated half-life extension moiety
DTHFPCIKFCRK

SEQ ID NO: 212 - protein, 11 aa, synthetic construct
  REGION 1..11: note = Made in Lab - hepcidin analogue
  MOD_RES 8: note = D-form lysine
  SITE 8: note = MISC_FEATURE - IsoGlu-Palm conjugated half-life extension moiety
  MOD_RES 9: note = N-Methyl-Phenylalanine
DTHFPCIKXGC

SEQ ID NO: 213 - protein, 10 aa, synthetic construct
  REGION 1..10: note = Made in Lab - hepcidin analogue
  MOD_RES 8: note = D-form lysine
  SITE 8: note = MISC_FEATURE - IsoGlu-Palm conjugated half-life extension moiety
DTHFPCIKFC

SEQ ID NO: 214 - protein, 10 aa, synthetic construct
  REGION 1..10: note = Made in Lab - hepcidin analogue
  SITE 8: note = MISC_FEATURE - IsoGlu-Palm conjugated half-life extension moiety
  MOD_RES 9: note = Beta-homophenylalanine
DTHFPCIKXC

SEQ ID NO: 215 - protein, 10 aa, synthetic construct
  REGION 1..10: note = Made in Lab - hepcidin analogue
  SITE 8: note = MISC_FEATURE - IsoGlu-Palm conjugated half-life extension moiety
  MOD_RES 9: note = Alpha- Methylphenylalanine
DTHFPCIKXC

SEQ ID NO: 216 - protein, 10 aa, synthetic construct
  REGION 1..10: note = Made in Lab - hepcidin analogue
  MOD_RES 4: note = Beta,Beta-diphenylalanine
  SITE 8: note = MISC_FEATURE - IsoGlu-Palm conjugated half-life extension moiety
  MOD_RES 9: note = Alpha- Methylphenylalanine
DTHXPCIKXC

SEQ ID NO: 217 - protein, 10 aa, synthetic construct
  REGION 1..10: note = Made in Lab - hepcidin analogue
  MOD_RES 4: note = Alpha-Methyl Phenylalanine
  SITE 8: note = MISC_FEATURE - IsoGlu-Palm conjugated half-life extension moiety
  MOD_RES 9: note = Alpha- Methylphenylalanine
DTHXPCIKXC

SEQ ID NO: 218 - protein, 10 aa, synthetic construct
  REGION 1..10: note = Made in Lab - hepcidin analogue
  MOD_RES 4: note = N-Methyl Phenylalanine
  SITE 8: note = MISC_FEATURE - IsoGlu-Palm conjugated half-life extension moiety
  MOD_RES 9: note = Alpha- Methylphenylalanine
DTHXPCIKXC

SEQ ID NO: 219 - protein, 10 aa, synthetic construct
  REGION 1..10: note = Made in Lab - hepcidin analogue
  MOD_RES 4: note = Beta-homophenylalanine
  SITE 8: note = MISC_FEATURE - IsoGlu-Palm conjugated half-life extension moiety
  MOD_RES 9: note = Alpha- Methylphenylalanine
DTHXPCIKXC

SEQ ID NO: 220 - protein, 10 aa, synthetic construct
  REGION 1..10: note = Made in Lab - hepcidin analogue
  SITE 8: note = MISC_FEATURE - IsoGlu-Palm conjugated half-life extension moiety
  MOD_RES 9: note = Alpha- Methylphenylalanine
DTHWPCIKXC

SEQ ID NO: 221 - protein, 10 aa, synthetic construct
  REGION 1..10: note = Made in Lab - hepcidin analogue
  MOD_RES 5: note = Nipecotic acid
  SITE 8: note = MISC_FEATURE - IsoGlu-Palm conjugated half-life extension moiety
  MOD_RES 9: note = Alpha- Methylphenylalanine
DTHFXCIKXC

SEQ ID NO: 222 - protein, 10 aa, synthetic construct
  REGION 1..10: note = Made in Lab - hepcidin analogue
  SITE 8: note = MISC_FEATURE - PEG11-Palm conjugated half-life extension moiety
DTHFPCIKFC

SEQ ID NO: 223 - protein, 10 aa, synthetic construct
  REGION 1..10: note = Made in Lab - hepcidin analogue
  SITE 8: note = MISC_FEATURE - isoGlu-Palm conjugated half-life extension moiety
DTHFPCIKFC

SEQ ID NO: 224 - protein, 11 aa, synthetic construct
  REGION 1..11: note = Made in Lab - hepcidin analogue
  MOD_RES 8: note = D-form lysine
  SITE 8: note = MISC_FEATURE - PEG11-Palm conjugated half-life extension moiety
DTHFPCIKFKC

SEQ ID NO: 225 - protein, 11 aa, synthetic construct
  REGION 1..11: note = Made in Lab - hepcidin analogue
  MOD_RES 8: note = D-form lysine
  SITE 8: note = MISC_FEATURE - PEG11-Palm conjugated half-life extension moiety
  MOD_RES 10: note = D-form lysine
DTHFPCIKFKC

SEQ ID NO: 226 - protein, 11 aa, synthetic construct
  REGION 1..11: note = Made in Lab - hepcidin analogue
  MOD_RES 8: note = D-form lysine
  SITE 8: note = MISC_FEATURE - PEG11-Palm conjugated half-life extension moiety
  MOD_RES 10: note = D-form arginine
DTHFPCIKFRC

SEQ ID NO: 227 - protein, 11 aa, synthetic construct
  REGION 1..11: note = Made in Lab - hepcidin analogue
  SITE 8: note = MISC_FEATURE - isoGlu-Palm conjugated half-life extension moiety
DTHFPCIKFKC

SEQ ID NO: 228 - protein, 11 aa, synthetic construct
  REGION 1..11: note = Made in Lab - hepcidin analogue
  MOD_RES 4: note = Beta,Beta-diphenylalanine
  SITE 8: note = MISC_FEATURE - PEG11-Palm conjugated half-life extension moiety
  MOD_RES 9: note = Beta-homophenylalanine
  MOD_RES 10: note = D-form lysine
DTHXPCIKXKC

SEQ ID NO: 229 - protein, 10 aa, synthetic construct
  REGION 1..10: note = Made in Lab - hepcidin analogue
  MOD_RES 4: note = Beta,Beta-diphenylalanine
  SITE 8: note = MISC_FEATURE - Ahx-Palm conjugated half-life extension moiety
  MOD_RES 9: note = Beta-homophenylalanine
DTHXPCIKXC

SEQ ID NO: 230 - protein, 11 aa, synthetic construct
  REGION 1..11: note = Made in Lab - hepcidin analogue
  MOD_RES 4: note = Beta,Beta-diphenylalanine
  SITE 8: note = MISC_FEATURE - Ahx-Palm conjugated half-life extension moiety
  MOD_RES 9: note = Beta-homophenylalanine
  MOD_RES 11: note = D-form lysine
DTHXPCIKXCK

SEQ ID NO: 231 - protein, 9 aa, synthetic construct
  REGION 1..9: note = Sythetic Construct - Dimer linked by K-K-isoGlu-Palm conjugated half-life meoiety
DTHFPCIKF

SEQ ID NO: 232 - protein, 9 aa, synthetic construct
  REGION 1..9: note = Sythetic Construct - Dimer linked by dK-K-isoGlu-Palm conjugated half-life meoiety
DTHFPCIKF

SEQ ID NO: 233 - protein, 9 aa, synthetic construct
  REGION 1..9: note = Sythetic Construct - Dimer linked by K-isoGlu-Palm conjugated half-life meoiety
  MOD_RES 8: note = D-form lysine
DTHFPCIKF

SEQ ID NO: 234 - protein, 9 aa, synthetic construct
  REGION 1..9: note = Sythetic Construct - Dimer linked by K-K-isoGlu-Palm conjugated half-life moiety
  MOD_RES 9: note = Phe (4-OCH2CH2NH2)
DTHFPCIKX

SEQ ID NO: 235 - protein, 9 aa, synthetic construct
  REGION 1..9: note = Sythetic Construct - Dimer linked by K-K-isoGlu-Palm conjugated half-life meoiety
  MOD_RES 9: note = Alpha-Methylphenylalanine
DTHFPCIKX

SEQ ID NO: 236 - protein, 9 aa, synthetic construct
  REGION 1..9: note = Sythetic Construct - Dimer linked by IDA [(beta-alanine)-Palm] conjugated half-life meoiety
  MOD_RES 8: note = D-form lysine
DTHFPCIKF

SEQ ID NO: 237 - protein, 9 aa, synthetic construct
  REGION 1..9: note = Sythetic Construct - Dimer linked by IDA [(beta-alanine)-Palm] conjugated half-life meoiety
  MOD_RES 9: note = N-Methylphenylalanine
DTHFPCIKX

SEQ ID NO: 238 - protein, 9 aa, synthetic construct
  REGION 1..9: note = Sythetic Construct - Dimer linked by IDA [(beta-alanine)-Palm] conjugated half-life meoiety
  MOD_RES 9: note = Alpha-Methylphenylalanine
DTHFPCIKX

SEQ ID NO: 239 - protein, 10 aa, synthetic construct
  REGION 1..10: note = Sythetic Construct - Dimer linked by IDA [(beta-alanine)-Palm] conjugated half-life meoiety
  MOD_RES 10: note = D-form lysine
DTHFPCIIFK

SEQ ID NO: 240 - protein, 9 aa, synthetic construct
  REGION 1..9: note = Sythetic Construct - Dimer linked by K-K-isoGlu-Palm conjugated half-life moiety
  MOD_RES 8: note = D-form lysine
  MOD_RES 9: note = Alpha-Methylphenylalanine
DTHFPCIKX

SEQ ID NO: 241 - protein, 9 aa, synthetic construct
  REGION 1..9: note = Sythetic Construct - Dimer linked by K-K-isoGlu-Palm conjugated half-life moiety
  MOD_RES 4: note = Biphenylalanine
  MOD_RES 8: note = D-form lysine
DTHXPCIKF

SEQ ID NO: 242 - protein, 9 aa, synthetic construct
  REGION 1..9: note = Sythetic Construct - Dimer linked by K-K-isoGlu-Palm conjugated half-life moiety
  MOD_RES 9: note = Beta-homophenylalanine
DTHFPCIKX

SEQ ID NO: 243 - protein, 9 aa, synthetic construct
  REGION 1..9: note = Sythetic Construct - Dimer linked by K-K-isoGlu-Palm conjugated half-life moiety
  MOD_RES 9: note = Beta-homophenylalanine
DTHFPCIKX

SEQ ID NO: 244 - protein, 9 aa, synthetic construct
  REGION 1..9: note = Sythetic Construct - Dimer linked by IDA [(beta-alanine)-Palm] conjugated half-life meoiety
  MOD_RES 8: note = D-form lysine
  MOD_RES 9: note = N-Methylphenylalanine
DTHFPCIKX

SEQ ID NO: 245 - protein, 9 aa, synthetic construct
  REGION 1..9: note = Sythetic Construct - Dimer linked by IDA [(beta-alanine)-Palm] conjugated half-life meoiety
  MOD_RES 4: note = Biphenylalanine
  MOD_RES 8: note = D-form lysine
  MOD_RES 9: note = N-Methylphenylalanine
DTHXPCIKX

SEQ ID NO: 246 - protein, 9 aa, synthetic construct
  REGION 1..9: note = Sythetic Construct - Dimer linked by IDA [(beta-alanine)-Palm] conjugated half-life meoiety
  MOD_RES 9: note = Beta-homophenylalanine
DTHFPCIKX

SEQ ID NO: 247 - protein, 9 aa, synthetic construct
  REGION 1..9: note = Sythetic Construct - Dimer linked by IDA [(beta-alanine)-Palm] conjugated half-life meoiety
  MOD_RES 8: note = D-form lysine
  MOD_RES 9: note = Beta-homophenylalanine
DTHFPCIKX

SEQ ID NO: 248 - protein, 9 aa, synthetic construct
  REGION 1..9: note = Sythetic Construct - Dimer linked by IDA [(beta-alanine)-Palm] conjugated half-life meoiety
  MOD_RES 5: note = Nipecotic acid
  MOD_RES 8: note = D-form lysine
  MOD_RES 9: note = N-Methylphenylalanine
DTHFXCIKX

SEQ ID NO: 249 - protein, 4 aa, synthetic construct
  REGION 1..4: note = Made in Lab - peptide insert
PRSK

SEQ ID NO: 250 - protein, 5 aa, synthetic construct
  REGION 1..5: note = Made in Lab - peptide insert
  MOD_RES 5: note = sarcosine
PRSKX

SEQ ID NO: 251 - protein, 5 aa, synthetic construct
  REGION 1..5: note = Made in Lab - peptide insert
PRSKG

SEQ ID NO: 252 - protein, 17 aa, synthetic construct
  REGION 1..17: note = Made in Lab - hepcidin analogue
DTHFPCIKFEPRSKGCK

SEQ ID NO: 253 - protein, 4 aa, synthetic construct
  REGION 1..4: note = Made in Lab - peptide insert
PRSC

SEQ ID NO: 254 - protein, 5 aa, synthetic construct
  REGION 1..5: note = Made in Lab - peptide insert
PRSKC

SEQ ID NO: 255 - protein, 6 aa, synthetic construct
  REGION 1..6: note = Made in Lab - peptide insert
PRSKCK

SEQ ID NO: 256 - protein, 25 aa, Homo sapiens
DTHFPICIFCCGCCHRSKCGMCCKT

SEQ ID NO: 257 - protein, 9 aa, Homo sapiens
DTHFPICIF

SEQ ID NO: 258 - protein, 9 aa, synthetic construct
  REGION 1..9: note = Made in Lab - hepcidin analogue
  MOD_RES 1: note = D-form phenylalanine
  MOD_RES 2: note = D-form isoleucine
  MOD_RES 3: note = D-form cysteine
  MOD_RES 4: note = D-form isoleucine
  MOD_RES 5: note = D-form proline
  MOD_RES 6: note = D-form phenylalanine
  MOD_RES 7: note = D-form histidine
  MOD_RES 8: note = D-form threonine
  MOD_RES 9: note = D-form aspartic acid
FICIPFHTD